European Patent Application EP 4 365 192 A1, published May 8, 2024. Title: Microbial production of growth factors. Applicant: DSM IP Assets B.V. Application EP. The sequence listing filed with the application follows.

SEQUENCE LISTING (33 sequences)

SEQ ID NO: 1 - DNA, 1449 bp, KanMX selection with TEF1promoter and TEF1 terminator
  source 1..1449: mol_type = unassigned DNA
agatctgtttagcttgcctcgtccccgccgggtcacccggccagcgacatggaggcccagaataccctccttgacagtcttgacgtgcgcagctcaggggcatgatgtgactgtcgcccgtacatttagcccatacatccccatgtataatcatttgcatccatacattttgatggccgcacggcgcgaagcaaaaattacggctcctcgctgcagacctgcgagcagggaaacgctcccctcacagacgcgttgaattgtccccacgccgcgcccctgtagagaaatataaaaggttaggatttgccactgaggttcttctttcatatacttccttttaaaatcttgctaggatacagttctcacatcacatccgaacataaacaaccatgggtaaggaaaagactcacgtttcgaggccgcgattaaattccaacatggatgctgatttatatgggtataaatgggctcgcgataatgtcgggcaatcaggtgcgacaatctatcgattgtatgggaagcccgatgcgccagagttgtttctgaaacatggcaaaggtagcgttgccaatgatgttacagatgagatggtcagactaaactggctgacggaatttatgcctcttccgaccatcaagcattttatccgtactcctgatgatgcatggttactcaccactgcgatccccggcaaaacagcattccaggtattagaagaatatcctgattcaggtgaaaatattgttgatgcgctggcagtgttcctgcgccggttgcattcgattcctgtttgtaattgtccttttaacagcgatcgcgtatttcgtctcgctcaggcgcaatcacgaatgaataacggtttggttgatgcgagtgattttgatgacgagcgtaatggctggcctgttgaacaagtctggaaagaaatgcataagcttttgccattctcaccggattcagtcgtcactcatggtgatttctcacttgataaccttatttttgacgaggggaaattaataggttgtattgatgttggacgagtcggaatcgcagaccgataccaggatcttgccatcctatggaactgcctcggtgagttttctccttcattacagaaacggctttttcaaaaatatggtattgataatcctgatatgaataaattgcagtttcatttgatgctcgatgagtttttctaatcagtactgacaataaaaagattcttgttttcaagaacttgtcatttgtatagtttttttatattgtagttgttctattttaatcaaatgttagcgtgatttatattttttttcgcctcgacatcatctgcccagatgcgaagttaagtgcgcagaaagtaatatcatgcgtcaatcgtatgtgaatgctggtcgctatactgctgtcgattcgatactaacgccgccatccagtgtcgaaaacgagctc

SEQ ID NO: 2 - DNA, 4893 bp, CAS9 expression cassette GAP1 promoter and CYC1 terminator
  source 1..4893: mol_type = unassigned DNA
gatccttttttgtagaaatgtcttggtgtcctcgtccaatcaggtagccatctctgaaatatctggctccgttgcaactccgaacgacctgctggcaacgtaaaattctccggggtaaaacttaaatgtggagtaatggaaccagaaacgtctcttcccttctctctccttccaccgcccgttaccgtccctaggaaattttactctgctggagagcttcttctacggcccccttgcagcaatgctcttcccagcattacgttgcgggtaaaacggaggtcgtgtacccgacctagcagcccagggatggaaaagtcccggccgtcgctggcaataatagcgggcggacgcatgtcatgagattattggaaaccaccagaatcgaatataaaaggcgaacacctttcccaattttggtttctcctgacccaaagactttaaatttaatttatttgtccctatttcaatcaattgaacaactatcaaaacacatggacaagaagtactccattgggctcgatatcggcacaaacagcgtcggttgggccgtcattacggacgagtacaaggtgccgagcaaaaaattcaaagttctgggcaataccgatcgccacagcataaagaagaacctcattggcgccctcctgttcgactccggggagacggccgaagccacgcggctcaaaagaacagcacggcgcagatatacccgcagaaagaatcggatctgctacctgcaggagatctttagtaatgagatggctaaggtggatgactctttcttccataggctggaggagtcctttttggtggaggaggataaaaagcacgagcgccacccaatctttggcaatatcgtggacgaggtggcgtaccatgaaaagtacccaaccatatatcatctgaggaagaagcttgtagacagtactgataaggctgacttgcggttgatctatctcgcgctggcgcatatgatcaaatttcggggacacttcctcatcgagggggacctgaacccagacaacagcgatgtcgacaaactctttatccaactggttcagacttacaatcagcttttcgaagagaacccgatcaacgcatccggagttgacgccaaagcaatcctgagcgctaggctgtccaaatcccggcggctcgaaaacctcatcgcacagctccctggggagaagaagaacggcctgtttggtaatcttatcgccctgtcactcgggctgacccccaactttaaatctaacttcgacctggccgaagatgccaagcttcaactgagcaaagacacctacgatgatgatctcgacaatctgctggcccagatcggcgaccagtacgcagacctttttttggcggcaaagaacctgtcagacgccattctgctgagtgatattctgcgagtgaacacggagatcaccaaagctccgctgagcgctagtatgatcaagcgctatgatgagcaccaccaagacttgactttgctgaaggcccttgtcagacagcaactgcctgagaagtacaaggaaattttcttcgatcagtctaaaaatggctacgccggatacattgacggcggagcaagccaggaggaattttacaaatttattaagcccatcttggaaaaaatggacggcaccgaggagctgctggtaaagcttaacagagaagatctgttgcgcaaacagcgcactttcgacaatggaagcatcccccaccagattcacctgggcgaactgcacgctatcctcaggcggcaagaggatttctacccctttttgaaagataacagggaaaagattgagaaaatcctcacatttcggataccctactatgtaggccccctcgcccggggaaattccagattcgcgtggatgactcgcaaatcagaagagaccatcactccctggaacttcgaggaagtcgtggataagggggcctctgcccagtccttcatcgaaaggatgactaactttgataaaaatctgcctaacgaaaaggtgcttcctaaacactctctgctgtacgagtacttcacagtttataacgagctcaccaaggtcaaatacgtcacagaagggatgagaaagccagcattcctgtctggagagcagaagaaagctatcgtggacctcctcttcaagacgaaccggaaagttaccgtgaaacagctcaaagaagactatttcaaaaagattgaatgtttcgactctgttgaaatcagcggagtggaggatcgcttcaacgcatccctgggaacgtatcacgatctcctgaaaatcattaaagacaaggacttcctggacaatgaggagaacgaggacattcttgaggacattgtcctcacccttacgttgtttgaagatagggagatgattgaagaacgcttgaaaacttacgctcatctcttcgacgacaaagtcatgaaacagctcaagaggcgccgatatacaggatgggggcggctgtcaagaaaactgatcaatgggatccgagacaagcagagtggaaagacaatcctggattttcttaagtccgatggatttgccaaccggaacttcatgcagttgatccatgatgactctctcacctttaaggaggacatccagaaagcacaagtttctggccagggggacagtcttcacgagcacatcgctaatcttgcaggtagcccagctatcaaaaagggaatactgcagaccgttaaggtcgtggatgaactcgtcaaagtaatgggaaggcataagcccgagaatatcgttatcgagatggcccgagagaaccaaactacccagaagggacagaagaacagtagggaaaggatgaagaggattgaagagggtataaaagaactggggtcccaaatccttaaggaacacccagttgaaaacacccagcttcagaatgagaagctctacctgtactacctgcagaacggcagggacatgtacgtggatcaggaactggacatcaatcggctctccgactacgacgtggatcatatcgtgccccagtcttttctcaaagatgattctattgataataaagtgttgacaagatccgataaaaatagagggaagagtgataacgtcccctcagaagaagttgtcaagaaaatgaaaaattattggcggcagctgctgaacgccaaactgatcacacaacggaagttcgataatctgactaaggctgaacgaggtggcctgtctgagttggataaagccggcttcatcaaaaggcagcttgttgagacacgccagatcaccaagcacgtggcccaaattctcgattcacgcatgaacaccaagtacgatgaaaatgacaaactgattcgagaggtgaaagttattactctgaagtctaagctggtctcagatttcagaaaggactttcagttttataaggtgagagagatcaacaattaccaccatgcgcatgatgcctacctgaatgcagtggtaggcactgcacttatcaaaaaatatcccaagcttgaatctgaatttgtttacggagactataaagtgtacgatgttaggaaaatgatcgcaaagtctgagcaggaaataggcaaggccaccgctaagtacttcttttacagcaatattatgaattttttcaagaccgagattacactggccaatggagagattcggaagcgaccacttatcgaaacaaacggagaaacaggagaaatcgtgtgggacaagggtagggatttcgcgacagtccggaaggtcctgtccatgccgcaggtgaacatcgttaaaaagaccgaagtacagaccggaggcttctccaaggaaagtatcctcccgaaaaggaacagcgacaagctgatcgcacgcaaaaaagattgggaccccaagaaatacggcggattcgattctcctacagtcgcttacagtgtactggttgtggccaaagtggagaaagggaagtctaaaaaactcaaaagcgtcaaggaactgctgggcatcacaatcatggagcgatcaagcttcgaaaaaaaccccatcgactttctcgaggcgaaaggatataaagaggtcaaaaaagacctcatcattaagcttcccaagtactctctctttgagcttgaaaacggccggaaacgaatgctcgctagtgcgggcgagctgcagaaaggtaacgagctggcactgccctctaaatacgttaatttcttgtatctggccagccactatgaaaagctcaaagggtctcccgaagataatgagcagaagcagctgttcgtggaacaacacaaacactaccttgatgagatcatcgagcaaataagcgaattctccaaaagagtgatcctcgccgacgctaacctcgataaggtgctttctgcttacaataagcacagggataagcccatcagggagcaggcagaaaacattatccacttgtttactctgaccaacttgggcgcgcctgcagccttcaagtacttcgacaccaccatagacagaaagcggtacacctctacaaaggaggtcctggacgccacactgattcatcagtcaattacggggctctatgaaacaagaatcgacctctctcagctcggtggagacagcagggctgaccccaagaagaagaggaaggtgtgatctcttctcgagtcatgtaattagttatgtcacgcttacattcacgccctccccccacatccgctctaaccgaaaaggaaggagttagacaacctgaagtctaggtccctatttatttttttatagttatgttagtattaagaacgttatttatatttcaaatttttcttttttttctgtacagacgcgtgtacgcatgtaacattatactgaaaaccttgcttgagaaggttttgggacgctcgaaggctttaatttgcgg

SEQ ID NO: 3 - DNA, 478 bp, gRNA LIG4_1
  source 1..478: mol_type = unassigned DNA
atgctatacgaacggtagaattcgatatcagatccactagtggcctatgcggccgccaccaagtatcacagttggattaattagatatgaaaactaattgtttatttacaataagacgcagatagcccctttcgttcagaatagtcatttcatcatatttcctgatatatatgtctacattagtcttcaattgaactctgtcacagtggccgagtggttaaggcgatgccctgctattctttgaaagtagttaaggcattgggttctacctgcgcaggttcgaatcctgtctgtgacggtgttctagataaagtacccgttttagagctagaaatagcaagttaaaataaggctagtccgttatcaacttgaaaaagtggcaccgagtcggtggtgctttttttgttttttatgtctcggtggagctccagcttttgttccctttagtgagggttaattgcgcgcttggcgtaatcat

SEQ ID NO: 4 - DNA, 20 bp, primer pCASPP-01
  source 1..20: mol_type = unassigned DNA
cgcgcttggcgtaatcatgg

SEQ ID NO: 5 - DNA, 21 bp, primer pCASPP-01
  source 1..21: mol_type = unassigned DNA
cataggccactagtggatctg

SEQ ID NO: 6 - DNA, 31 bp, primer gRNA
  source 1..31: mol_type = unassigned DNA
atgctatacgaacggtagaattcgatatcag

SEQ ID NO: 7 - DNA, 28 bp, Primer gRNA
  source 1..28: mol_type = unassigned DNA
atgattacgccaagcgcgcaattaaccc

SEQ ID NO: 8 - DNA, 101 bp, LIG4_1 repair DNA
  source 1..101: mol_type = unassigned DNA
tacaactcctcatgactggggatcagaatttcaacttgatttgccgctaattaaaaataatgatttacatttaagaagtaacagcacatatatactgtaag

SEQ ID NO: 9 - DNA, 20 bp, Primer check lig4 deletion
  source 1..20: mol_type = unassigned DNA
gtgctagagggtgctcttgg

SEQ ID NO: 10 - DNA, 20 bp, Primer check lig4 deletion
  source 1..20: mol_type = unassigned DNA
aacgtgtggttaccaaggct

SEQ ID NO: 11 - protein, 155 aa, FGF301
MAAGSITTLPALPEDGGSGAFPPGHFKDPKRLYCKNGGFFLRIHPDGRVDGVREKSDPHIKLQLQAEERGVVSIKGVCANRYLAMKEDGRLLASKCVTDECFFFERLESNNYNTYRSRKYSSWYVALKRTGQYKLGPKTGPGQKAILFLPMSAKS

SEQ ID NO: 12 - protein, 133 aa, FGF320
MANYKKPKLLYCSNGGHFLRIHPDGRVDGVREKSDPHIKLQLQAEERGVVSIKGVCANRYLAMDTSGLLYGSQTPSEECLFLERLEENHYNTYTSKKHAEKNWFVGLKKNGSCKRGPRTHYGQKAILFLPLPV

SEQ ID NO: 13 - protein, 133 aa, FGF321
MANYKKPKLLYSSNGGHFLRIHPDGRVDGVREKSDPHIKLQLQAEERGVVSIKGVCANRYLCMDTSGLLYGSQTPSEECLFLERLEENHYNTYTSKKHAEKNWFVGLKKNGSAKRGPRTHYGQKAILFLPLPV

SEQ ID NO: 14 - protein, 133 aa, FGF322
MANYKKPKLLYCSNGGHFLRIHPDGRVDGVREKSDPHIKLQLIAEERGVVSIKGVCANRYLAMDTSGLLYGSQTPSEECLFLERLEENGYNTYTSKKHAEKNWFVGLTKNGSCKRGPRTHYGQKAILFLPLPV

SEQ ID NO: 15 - protein, 133 aa, FGF323
MANYKKPKLLYSSNGGHFLRIHPDGRVDGVREKSDPHIKLQLIAEERGVVSIKGVCANRYLCMDTSGLLYGSQTPSEECLFLERLEENGYNTYTSKKHAEKNWFVGLKKNGSAKRGPRTHYGQKAILFLPLPV

SEQ ID NO: 16 - DNA, 468 bp, FGF301
  source 1..468: mol_type = unassigned DNA
atggctgctggttccattaccactttgccagctttgccagaagatggtggttctggtgctttcccaccaggtcacttcaaggacccaaagagattatactgtaagaacggtggtttctttttgagaattcacccagacggtcgtgtcgacggtgtcagagaaaaatctgaccctcacatcaagttgcaattacaagctgaagaaagaggtgttgtttccatcaagggtgtttgtgccaaccgttacttggctatgaaggaagatggtagattgttggcttccaagtgtgtcaccgatgaatgtttcttcttcgaaagattggaatctaacaactacaacacctacagatccagaaagtactcttcttggtacgttgctttgaagagaactggtcaatacaaattgggtccaaagactggtccaggtcaaaaggccatcttattcttgccaatgtctgccaagtcctaa

SEQ ID NO: 17 - DNA, 402 bp, FGF320
  source 1..402: mol_type = unassigned DNA
atggctaactacaagaagccaaaattgttgtactgttccaacggtggtcacttcttgagaattcacccagatggtcgtgtcgatggtgtcagagaaaaatctgaccctcacatcaagttgcaattacaagctgaagaaagaggtgttgtttccatcaagggtgtttgtgccaacagatacttggctatggacacttctggtttgttgtacggttctcaaaccccatctgaagaatgtttgttcttggaaagattggaagaaaaccattacaacacttacacttctaagaagcacgctgaaaagaactggttcgtcggtttgaagaagaacggttcttgtaagagaggtccaagaacccactacggtcaaaaggccatcttattcttgccattaccagtttaa

SEQ ID NO: 18 - DNA, 402 bp, FGF321
  source 1..402: mol_type = unassigned DNA
atggctaactacaagaagccaaaattgttgtactcttccaacggtggtcacttcttgagaattcacccagatggtcgtgtcgatggtgtcagagaaaaatctgaccctcacatcaagttgcaattacaagctgaagaaagaggtgttgtttccatcaagggtgtttgtgccaacagatacttgtgtatggacacttctggtttgttgtacggttctcaaaccccatctgaagaatgtttgttcttggaaagattggaagaaaaccattacaacacttacacttctaagaagcacgctgaaaagaactggttcgtcggtttgaagaagaacggttctgctaagagaggtccaagaacccactacggtcaaaaggccatcttattcttgccattaccagtttaa

SEQ ID NO: 19 - DNA, 402 bp, FGF322
  source 1..402: mol_type = unassigned DNA
atggctaactacaagaagccaaaattgttgtactgttccaacggtggtcacttcttgagaattcacccagatggtcgtgtcgatggtgtcagagaaaaatctgaccctcacatcaagttgcaattaatcgctgaagaaagaggtgttgtttccatcaagggtgtttgtgccaacagatacttggctatggacacttctggtttgttgtacggttctcaaaccccatctgaagaatgtttgttcttggaaagattggaagaaaacggttacaacacttacacttctaagaagcacgctgaaaagaactggttcgtcggtttgaccaagaacggttcttgtaagagaggtccaagaacccactacggtcaaaaggccatcttattcttgccattaccagtttaa

SEQ ID NO: 20 - DNA, 402 bp, FGF323
  source 1..402: mol_type = unassigned DNA
atggctaactacaagaagccaaaattgttgtactcttccaacggtggtcacttcttgagaattcacccagatggtcgtgtcgatggtgtcagagaaaaatctgaccctcacatcaagttgcaattaatcgctgaagaaagaggtgttgtttccatcaagggtgtttgtgccaacagatacttgtgtatggacacttctggtttgttgtacggttctcaaaccccatctgaagaatgtttgttcttggaaagattggaagaaaacggttacaacacttacacttctaagaagcacgctgaaaagaactggttcgtcggtttgaagaagaacggttctgctaagagaggtccaagaacccactacggtcaaaaggccatcttattcttgccattaccagtttaa

SEQ ID NO: 21 - DNA, 523 bp, Opol promoter
  source 1..523: mol_type = unassigned DNA
cggtctcggtgcgagatcccaccgcgttcctgggtaccgggacgtgaggcagcgcgacatccatcaaatataccaggcgccaaccgagtctctcggaaaacagcttctggatatcttccgctggcggcgcaacgacgaataatagtccctggaggtgacggaatatatatgtgtggagggtaaatctgacagggtgtagcaaaggtaatattttcctaaaacatgcaatcggctgccccgcaacgggaaaaagaatgactttggcactcttcaccagagtggggtgtcccgctcgtgtgtgcaaataggctcccactggtcaccccggattttgcagaaaaacagcaagttccggggtgtctcactggtgtccgccaataagaggagccggcaggcacggagtctacatcaagctgtctccgatacactcgactaccatccggctctctcagagaggggaatggcactataaataccgcctccttgcgctctctgccttcatcaatcaaataatgggagaccg

SEQ ID NO: 22 - DNA, 269 bp, AOX1 terminator
  source 1..269: mol_type = unassigned DNA
cggtctcgtaaacaagaggatgtcagaatgccatttgcctgagagatgcaggcttcatttttgatacttttttatttgtaacctatatagtataggattttttttgtcattttgtttcttctcgtacgagcttgctcctgatcagcctatctcgcagctgatgaatatcttgtggtaggggtttgggaaaatcattcgagtttgatgtttttcttggtatttcccactcctcttcagagtacagaagattaagtgagcctcggagaccg

SEQ ID NO: 23 - DNA, 50 bp, connector A
  source 1..50: mol_type = unassigned DNA
ttgcccatcgaacgtacaagtactcctctgttctctccttcctttgcttt

SEQ ID NO: 24 - DNA, 50 bp, connector B
  source 1..50: mol_type = unassigned DNA
cggatcgatgtacacaaccgactgcacccaaacgaacacaaatcttagca

SEQ ID NO: 25 - DNA, 50 bp, connector C
  source 1..50: mol_type = unassigned DNA
acgctttccggcatcttccagaccacagtatatccatccgcctcctgttg

SEQ ID NO: 26 - DNA, 120 bp, Pp_pTEFUP_FLANK5.acc - a (100bp flank)
  source 1..120: mol_type = unassigned DNA
accagtaacacgcttaaggtttggaacaacactaaactaccttgcggtactaccattgacactacacatccttaattccaatcctgtctggcctccttcattgcccatcgaacgtacaag

SEQ ID NO: 27 - DNA, 23 bp, Reverse connector b
  source 1..23: mol_type = unassigned DNA
tgctaagatttgtgttcgtttgg

SEQ ID NO: 28 - DNA, 123 bp, c - Pp_pTEFUP_FLANK3.acc (100bp flank)
  source 1..123: mol_type = unassigned DNA
gcgacagttattacctgattgggttaaagatttaaaattttttttttttcacttgatacgcaatctgacacgagttggaatgggcaagatggttaaaaggcaacaggaggcggatggatatac

SEQ ID NO: 29 - DNA, 20 bp, Forward connector b
  source 1..20: mol_type = unassigned DNA
cggatcgatgtacacaaccg

SEQ ID NO: 30 - DNA, 20 bp, Primer pTEFUP check fw
  source 1..20: mol_type = unassigned DNA
acttgacccgtcatacaggc

SEQ ID NO: 31 - DNA, 21 bp, Primer conA rev
  source 1..21: mol_type = unassigned DNA
aaagcaaaggaaggagagaac

SEQ ID NO: 32 - DNA, 21 bp, Primer conC forw
  source 1..21: mol_type = unassigned DNA
acgctttccggcatcttccag

SEQ ID NO: 33 - DNA, 20 bp, Primer pTEFUP check rv
  source 1..20: mol_type = unassigned DNA
gccaatcatgtacgagtgcg